European Patent Application EP 4 219 545 A1, published August 2, 2023. Title: Method for Decreasing Immunogenicity. Applicant: Novartis AG. Application EP. The sequence listing filed with the application follows.

SEQUENCE LISTING (4 sequences)

SEQ ID NO: 1 - protein, 251 aa, synthetic construct
  REGION 1..251: note = antibody fragment
EIVMTQSPSTLSASVGDRVIITCQASEIIHSWLAWYQQKPGKAPKLLIYLASTLASGVPSRFSGSGSGAEFTLTISSLQPDDFATYYCQNVYLASTNGANFGQGTKLTVLGGGGGSGGGGSGGGGSGGGGSEVQLVESGGGLVQPGGSLRLSCTASGFSLTDYYYMTWVRQAPGKGLEWVGFIDPDDDPYYATWAKGRFTISRDTSKNTVYLQMNSLRAEDTAVYYCAGGDHNSGWGLDIWGQGTLVTVSS

SEQ ID NO: 2 - protein, 254 aa, synthetic construct
  REGION 1..254: note = antibody fragment
MEIVMTQSPSTLSASLGDRVIITCQSSQSVYGNIWMAWYQQKSGKAPKLLIYQASKLASGVPSRFSGSGSGAEFSLTISSLQPDDFATYYCQGNFNTGDRYAFGQGTKLTVLGGGGGSGGGGSGGGGSGGGGSEVQLVESGGGLVQPGGSLRLSCTASGFTISRSYWICWVRQAPGKGLEWVACIYGDNDITPLYANWAKGRFPVSTDTSKNTVYLQMNSLRAEDTAVYYCARLGYADYAYDLWGQGTLVTVSS

SEQ ID NO: 3 - protein, 245 aa, synthetic construct
  REGION 1..245: note = antibody fragment
DIVMTQSPSSLSASVGDRVTLTCTASQSVSNDVVWYQQRPGKAPKLLIYSAFNRYTGVPSRFSGRGYGTDFTLTISSLQPEDVAVYYCQQDYNSPRTFGQGTKLEVKRGGGGSGGGGSGGGGSSGGGSQVQLVQSGAEVKKPGASVKVSCTASGYTFTHYGMNWVRQAPGKGLEWMGWINTYTGEPTYADKFKDRFTFSLETSASTVYMELTSLTSDDTAVYYCARERGDAMDYWGQGTLVTVSS

SEQ ID NO: 4 - protein, 251 aa, synthetic construct
  REGION 1..251: note = antibody fragment
EIVMTQSPSTLSASVGDRVIITCQASEIIHSWLAWYQQKPGKAPKLLIYLASTLASGVPSRFSGSGSGAEFTLTISSLQPDDFATYYCQNVYLASTNGANFGQGTKLTVLGGGGGSGGGGSGGGGSGGGGSEVQLVESGGGSVQPGGSLRLSCTASGFSLTDYYYMTWVRQAPGKGLEWVGFIDPDDDPYYATWAKGRFTISRDTSKNTVYLQMNSLRAEDTATYYCAGGDHNSGWGLDIWGQGTTVTVSS